European Patent Application EP 4 388 877 A1, published June 26, 2024. Title: Microorganism capable of forming a metabolic biofilm and methods for producing the same and of using it. Applicant: BRAIN Biotech AG. The sequence listing filed with the application follows.

SEQUENCE LISTING (2 sequences)

SEQ ID NO: 1 - DNA, 28 bp, synthetic construct
  misc_feature 1..28: note = groEL primer 60-A; groEL locus (Biosci Biotechnol Biochem.; 1992Dec;56(12):1995-2002; doi: 10.1271/bbb.56.1995)
  source 1..28: mol_type = other DNA
accctgggcccgagggccgcaacgtcgt

SEQ ID NO: 2 - DNA, 28 bp, synthetic construct
  misc_feature 1..28: note = groEL primer 160-B; groEL locus (Biosci Biotechnol Biochem.; 1992Dec;56(12):1995-2002; doi: 10.1271/bbb.56.1995)
  source 1..28: mol_type = other DNA
tgaccgcgacgccgcccgccagcttcgc